European Patent Specification EP 3 504 346 B1, published August 16, 2023. Title: Fecal Bacterial Markers for Colorectal Cancer. Applicant: The Chinese University of Hong Kong. The sequence listing filed with the application follows.

SEQUENCE LISTING (20 sequences)

SEQ ID NO: 1 - DNA, 1062 bp, Roseburia intestinalis
atggaaaaagtaaaggcattttgtaaacggaaaaacattgagatatccgtcaagcgctacctgattgatgcacttggtgcgatggcacagggattatttgcatcgcttttgatcggaacgatcatcagtacacttggaacgcagcttaatattccgattcttgtgacagtcgggacttacgcgaaagcggcagtcggaccggcaatggcgatcgcaatcggatatgcactgcaggcagcgcctttagtactgttttcacttgcggcagtcggtgcggcggcaaatgaacttggcggggcaggcggaccgcttgcggtacttgtggttgcaatttttgcagcagaatttggaaaagcagtttccaaagagacaaaaatcgatattattgtcactccgtttgtgaccatttttgtcggggtcgcgctttctatctggtgggctccggcgatcggtgcggcagcgagtgcagtcggtaatgcgatcatgtgggcaaccgagctgcagccgtttttcatgggaatcattgtatctgtgatcgtcgggattgcactgacactgccgatcagcagcgcagcaatctgtgcagcacttggactgaccggattagccggtggtgcagcacttgccggatgctgtgcgcagatggtcggatttgcagtggcaagtttccgtgaaaataaatggggcggattgtttgcacagggaatcggtacatccatgcttcagatgggtaatatcgtgaaaaatccgcgcatctggctgccggcgacattggcgtctgcaatcaccggaccgatcgcaatgtgtctgttccatttacagatgaatggtgcagcagtttcctccggtatgggaacctgtggactggtcggacagattggtgtctatacgggatggatcgcagatattgaagcgggaagcaaagctgccattacaccgatggactggatcggactgattttcgtaagctttcttctgccgggcgttttatcatggctttttagtgtgttattccgtaagatcggctggatcaaagaaggcgatatgaggctggacttataa

SEQ ID NO: 2 - DNA, 1161 bp, Bacteroides clarus
atgaaaatcaaacaattagcgaaaagcgcatcattcttgctggtggcaggttttatcagttttactattccgtcgtgtagcagtgaagaagaaatcatcatccttcaggatgtaaaagtaaacagtgaaagcttcaatctggccgaagacggcagtacgaccatagaagtcaaggtagtacccgaaaatactccaatagccaaagccgtactcagcacatcattatttaatgaaagcggtgttttcgaagtaacccgactcactcccaaaggtaacggtgtatggcagatagcagcaaaagtaaaggacttctcacgcattcaaaacggtcaggacgtaatactttccgtctatcaggaagataatatgtatatccaaaccacattgaaaataaacgacccatatagcatcgagggtaaatatacaccggtccatccgcaagcctttactttctacagtgccgaagacggcaaactgatggagattccgttcatcatcacagccgacaacgcagccgaccttgccgccatcagctacgacaatataaaggtagtcaatggcaccggaagctctacacccagcataagtatcacacatttcgcaatagctccgatgacaggtaaaacaggcttctatctgcaagtggataacgcccaactcgaaacggtaaaaaaagccatcacaaccatcgcttttttggactgccgggttatgataaccggccctaacggccgtgttgcctatactcctgtgcgcctcattgtttcttctccgaagtgcatcatcaaggacgaccaactcagcctgctgcatacagaattgtccgccccggagtttaatagacaaatcaccatagatatgacccacgatttttatcgtttgggcaaacagaatgataaaacaacctttgaggcgtttgaaaaccgaggcttgtataactcacaaggagaaatggcagatgcagaccctcagttcatttcgttgggttataccactcagggcaaaaatacaacatgtaacgtaactttaaaacatgatgccacaattcctgcaatcggcacttaccacatggtagaacgcctaaaaggatattgggaatatgacggaaagaaatatccgaccgtttgtacagacctgcaattccaaatcacgattaaataa

SEQ ID NO: 3 - DNA, 1935 bp, Lachnoclostridium sp.
aatatccgatatggcaacggagctctggtagtagtccgggcaagggaaaaccttgtacatggcgaagcagagcagattaccttcaatactaaaatattagaaaggtgcgtgaggcatttgagaaatccgattgaagtattgaaaactctacaagagaaagcaggcaacgagaactatcaatttgaacgcctgtaccgaaatctgtacaacgaggagtttttcctattggcatacggaaatctctctgcaaaagagggaaatctgaccaagggaacagacggcgccacaatagacggaatgggaatggagcggattcgcaagctgattgaaagcctgcggaaccacagttaccagccgtcccctgcgagacgtgcctatatcccaaaatctaatggaaaacggcgtccgttaggcataccctctgttgacgataagctggtgcaggaagttgtgaggttaattctcgaaagtgtgtatgaaagcaatttttctgaacattcgcatggttttagaccgaacaggagctgtcacacggcactgacccagattcaaagaaacttcacaggggttaaatggttcattgagggggacatcaaaggttattttgacaccatcgaccaccatatccttgtggatattttaagaaggcgcataaaggacgaatacctaatctcgctgatatggaaatttctgaaagccggatacttagaagactggaaattcaatcctacctattccggcactccgcaaggctcggtcatcagtccaatacttgccaatatctaccttaacgaattcgatacctatgttgaagaatacatagagaaattcaaccgtggtaaaagacgtgaaagaaacagtgagtatcgcttttatagtgatggcgcatcgaaactgagggtaaagtaccgcgggttatgggaaataatgacagccgatgaaaaagaaaaagccaaatgtgaagtaaatgagctcatgaaaaaagcaaaacagattccagctatgaatccgatggacagcaattaccgccgtctgctctattgcaggtatgcggatgattttatttgcggagtaatcggaagcaaggaagatgcagaaaccatcaaggctgattttagccggtacctgaaagaaaagctgggactggatatgtcggaagaaaagacactgattacacactcaaacgaaaaagcggcgttccttggctacgaaatcgctgtttccagaagcaatgaatacaaaaagataagcaacggacagaaggcaagaacctttaatgggcgtgttcatctatttatgccacataataaatgggttaagaagctgaccagttgcggagcaatggaaatcaaacagcaggacggcaaagaaatatggaaaccgcaggcgaggaaagacctcatcaacaaagagccgattgaaatcctaagcatttacaatgccgaaattcgtgggctgtacaattattattgtttggcaagcaacgtatgcaagctgcagaaatattactacatcatggaatacagcatgtaccagacgtttgcagcgaagtaccgtgataatttgcggaaaacgattaacaagcatacccgaaacggcgtgtttggtgtcagctacactacaaaaaccggcaacgagaaacgggcgacattcgtgaaaggaagcttccaaaaacggactgtcagcttagattacagtgatgaaatcccctcttatcctgccgcaaaatatagtcggaaaaacggcttaattgagcggttacagggtggaaaatgtgaactatgcggacagcagaccgacaatgtaaaagttcatcatgtcaggaagctgaaagaattagccggtatgaaagaatgggaaagaaaaatggttcagatgaacagaaaaactctggttgtttgtaatacatgttatggaaacataacaggcaagtaa

SEQ ID NO: 4 - DNA, 930 bp, Parvimonas micra
aatcaatttagaattggtttatcaagaatggagagagttgttagagaaagaatgtcaactcaagatccagaccttgctacgcctcaaggacttattaatataagacctcttgttgcgtctttaaaagaattcttcggttcttcacaattatcacaattcatggatcaaaacaatccacttgcagaacttactcataagagaagattatcagcattaggacctggtggtcttagtagagatagagcaggatacgaagtaagagacgttcatgaaagtcactacggaagaatttgtccgatagaaactccagaaggtccaaacatcggtcttattacttctcttacaacttatgcaagagttgatcaatatggatttattgaaacaccatatcgtgttgtaaataatggaattgctacaaaggacattgtttatttaactgctgatgaagaagatgaagttattatcgctcaagccaatgaaccacttgatgaaaatggacgttttgtaaacgaaagagtaagtggtcgtggtattaatggcgaaaatgatatttatccaagagatacaattcaacttatggacgtttctcctcaacaaattgtatcagttggtacagcaatgattcctttccttgaaaatgacgatgctactcgtgcgttgatgggttcaaacatgcaaagacaagcagtgcctctacttgttactgaagctcctattgtaggaaccggtatagaacataaagcggcaagagatagtggtgttgttatcattgctaaaaattcaggaattgttacaaaagttgatagtgatgaaattcatattaaaagagatttagataatgtagttgataaatatagattacttaaatttaaacgttcaaatcaaggaacaacaattaatcaaagacctatagttaatgaaaatgacaga

SEQ ID NO: 5 - DNA, 687 bp, Fusobacterium nucleatum
tctgcaaaagaaaaagttgctgcattagttgctgcattaaaagcagatggatatgattttactgttggtatccctcttgatacaccaataggaaaatctgaaagagttgtaagtgctggtaaagggattggagataaaaagaatatgaagctaattgaaaacttagcaaaacaagctggagcttctattggttcttctcgtccagtggcagaaacattgcaatatgtacctcttgaccgttatgtaggaatgtcaggacaaaaatttgttggaaacctttatatagcttgtggaatttcaggagctttacaacatttaaaaggaattaaagatgcaacaacaatagttgctataaatacaaactcaaatgctccaatatttaagaatgcagactatggaatagttggagatttagcagaaattttacctttattaactaaggaattagataatggagaagctaaaaaagatgcaccacctatgaagaaaatgaagagagttatacctagagtagtgtatagtcctcatgtatatgtatgtagtggttgtggacatgaatacaatcctgatttaggagatgaagattctgacataaaaccaggaactagatttaaagatttaccagaagattggacttgtcctgattgtggagatccaaaatctggatatatagatgcaaaaaaataa

SEQ ID NO: 6 - DNA, 627 bp, Clostridium hathewayi
atgcctatacttcagcagcttctcacattagtagagcagcacttcggtaacaaatgcgaaatcgtgcttcatgatctgacaaaggattacaaccataccattgtcgatatccgaaacggagacattacccatcgttccatcgggggctgcggaagcaacttagggctggaagtcctgcgcggaaccgtgctggatggggatcgttttaactatgttaccaccacacaggacggaaagattctccgttcctcatcgatctatctaaaaaatgatcagggcgaggtcatcggatcgatctgcgtgaacctggatatcacagagacacttcagtttgaagggtatttacgccagtttaaccagtttgacagctttacttccaacgacgaggagattttcgctcccgacgtgaataatcttctcagccatctgattcagatgggacaggaacagatcggaaagcctgcgctggagatgaacaagaacgagaagattgagtttatccgtttccttgaccagaaaggagcattcctcatcacgaagtccggggaacagatctgtgaacttctgggaatcagcaaatttaccttttataattaccttgaaagcagccgcagccagtcggattcg

SEQ ID NO: 7 - DNA, 1305 bp, m7
atgttagcaatcgtaggtttattaactatcctggtcgtaatgtttctgattatgacaaaaaaatgttcgactctggtcgcactgattgcagttcccatgattgcatgtgttattgtgggtcagggcgccgatatgggagggtacataacggccggtatcaaaagtgtggccgccaccggagtcatgtttatttttgcagtggcctttttcggtgtcatgggtgatgtgggtgcatttgaaatcgtagtgaataaaatactcaggattattgggaaagatcctttgaaaatctgtatcggcacgctgattatcacattgatgacccacctggacggctccggcgcaacgacatttttgatcacaataccggcgctgctgccgatatacgataaattgaagatggatcggcgtgtgctggcaactatagtggcggcaggagcaggaaccatgaatctcgtcccttggggagggccgacgatccgagcagcgacggcactggaggtctcactgaccgagctttacaatcctatgattgtccctcagctttgcggagtcgccgcctgcgtgacagtggcggtgatgtttggcctgaaggaacggaaacgtttaaaagggactctggaatctgtttcggtagagcctccgaaatttgaggacttaccggaggaggagagagtgaaacgccgtccccaccttgtctggtttaacattctgctcattatagttacaattgtgtcattggttatggagcttttgccgccggccggctgttttatggcggcgctgtgcatcgcaatgctggttaactaccgtgatttaaaggatcagggaaaacggatggacgagcatgcggtagcggccatgatgatggcatccaccctgtttggcgcaggctgctttaccggtatcctgggaggctgcggcatgctggaagcgatggcccagggactctgtgatattctcccggtagccattatgggtcacattgcgattttggtggcagttttctccatgcctctgtcgctgatgttcgatccggacagcttctactatgcagtacttccggtaattgcagtggcggccgaggtggccggtgttccggcattggcagtgggccgcgcggcgatatgcggacagattactgttggattccccatttcaccactgactccatccaccttccttctgacaggactaacgggcgtggatctcggggaccatcagaagcacagtttcgtgtggctgtggctgatttccctgacgattgtgctggttgccgtggtgatgggcgtaattccggtatag

SEQ ID NO: 8 - DNA, 504 bp, Unknown
atggttgcacttgtatggctactgattgaaatgaaatataaaatcagtgtcccatctccactgttgctcagcatggtttacaaacttttgcttccggctatgcctgcctatcttctggctaaaatcccctctgggaaattaacggccagcttgagaagaatgccgatttctacccatatcatgcttgtattgatcgtcatgctccgctttgcgccgactgtgctgcatgaatttggagaagtcagggaagccatgaaaattcgtggcttcttaaaatcggtcggtaatgttttgaggcatccaatggacacgttggaatacgccattgttccgatggtgttccgctccttaaagatcgcggacgagttagcagcttctgccatagtcaggggaattgaaagcccctacaagaaagaaagctactatgtcagccggatcgctgcgctggattactttttgattgttgtcagcgtgggagctgccgtgtgctgctgtcttttatag

SEQ ID NO: 9 - DNA, 750 bp, Ruminococcus obeum
atgaaaggaaaaagagttattgcaggcattctgcttgcaggaattttagcagttaccctggcagggtgtaaaaacacagataacactaaagaagaatcagaaaagccggttattaccctcggcagcgatagctatccaccatacaattatctgaatgaggatggtgtaccgacgggcatagatgtggaactagctacagaagctttcaaaagaatgggatatcaggtgaatgtcgtccaaatcaactgggaggagaaaaaagaactggtagagagtggaaagatcgattgtatcatgggttgtttttctatggaaggacgtcttgacgattaccgctgggcaggggcgtacatagcaagccgtcaggttgtagcggtaaatgaggacagtgatatttataaattgagtgaccttgagggaaagaacctggctgtccagtccacaactaaaccggaagttatatttctgaaccggttggataagagaatccacaaactgggaaatctgatcagtcttggacaccgcgagctgatatatacatttcttgggaaaggatatgtagatgcagttgccgcacatgaggaatcaatcatccagtatatgaaggattatgacatagacttccgtatcctggaagaatcgctgatgattacggggataggtgttgctttcgcaaaagatgatgacagaggaattgtgagcagatggaccagacccttgaagaaatgcgtaaggatggcacgtctttga

SEQ ID NO: 10 - DNA, 594 bp, Unknown
atggcaatgctcactgtagaaaatatcaatgtatattacggcgtgatccacgcccttaaagacatctcctttcaggtaaacgaaggcgagatcgtcgcactgatcggcgcaaacggtgccggcaaaaccaccaccctgcagactgtcagcggcatgctgagcgcaaagtccggttcgatccgatttcaggatcaggagatttccagaatgccggagcacaaaatcgtgaagcagggaatttcccacgtccccgaaggacgccggatgttctccaatctgacggttttggaaaacctgaaaatgggcgcttacaccagaaaagacaagcaggaaatcaacaattccctggaaatggtttatgagcggtttccccgcttaaaggaacgtacccgccagctggcaggaactctttccggcggtgaacagcagatgcttgcaatgggacgtgcactgatgtctcatccgaagatcatccttctggatgaaccgtctatgggactttcaccgatttttgtaaatgagattttcgaaattatcaagaaagtcagtgcagccggcacgaccgtacttctggtagagcagaatgcaaagaaa

SEQ ID NO: 11 - DNA, 708 bp, Unknown
gcagcttcaaactacgacctttgtacaacaatccttagaaatgaatggggatacgatggtatcgtaatgactgactggtgggccaagatgaacgacgttgtagaaggtggcgaagaatcaaatcaggatacaagagatatggttcgctcacagaacgacgtatatatggttgtaaacaataacggcgcagaagttaactcaaacaacgacaacacagagaaatcaattaaagagggaagacttacaatcggagaacttcagcgagctgcaatcaacatctgcaacttcattctttcagcacctgttattgaaagagaattagttgacacagacgttgcaaaacattacgattcagttccaaatgatcaggccaagtatgaagtatttaacattgaaaaagacaataaggtaatgttcaatagcggagcagaagcaacattggaagttgaagacgaaggggaatacacaattattgttaacatctcatttgacaagtccaacttatcacagtcaacagtaaacgttaatgccaacggcacaacaatggtagtaatccagactaatggaacagacggcaactggattacacagaagctttgcaaggttaaacttgacaagggtgtatacaacttaaaacttgaagaagtattagcaggaatcaaagttaaatatattcagtttaagaagattcctaagaaaaataaataa

SEQ ID NO: 12 - DNA, 1401 bp, Faecalibacterium prausnitzii
atgccgaacgaacgacattactccaatgaactgaatctggaaagcgtgggcatcaatctgccctacaacatgcaggccgagcagagcgtgctgggtgcggtgctgctcaagccggaaacactgaccgacctggttgagatcatccggccggaaatgttctacacccggcagaacgcccaaatttattcggaaatgctccggctgttcaccagcgaccagaccattgatttcgtcaccctgctggacgcggtcatctcagacggcgtgtttcccagcgcggacgaggcgaaagtctacctgaccggtctggccgagacggtgcccagcatctccaacgtgaaagcctacgcccagatcgtgcaggaaaaatatctggtccgccagctcatgggtgtggcgaaagatatcttgcaggatgcgggcgacgagccggacgcggacctgctgctggaaaacgccgagcagcgcatttatgagatccgctccgggcgggattccagcgccctgacgcccctttcttccagcatggtggaaacgctgaccaatctgcagaagatcagcggcccggatgccgataagtacaagggcatccctacaggcttccgcctgctggacaccgtgctcaccggccttggccgcggcgaccttattattctggctgcccgccccggtatgggcaagaccagttttgcgctgaacattgccacccgcgtggccatgcagcagaaagtaccggtggccatcttcagcctcgaaatgaccaaggagcagctgaccaaccggatcctctcggcggaggccggcatcgacagccaggcgttccgcaccggcgccctccgggcggaggactgggagtacctggcccttgccaccgagaagctccatgacgcgcccatttatatggatgacacctcgggcatcaccatcaccgagatgaaagccaagatccgccgggtgaaccaggaccccagccgccccaatgtggggctcatcgtcatcgactatctgcagctgatgaccacgggccagcgcaccgagaaccgtgtacaggagatcagctccatcacccgaaacctcaagatcatggccaaagagatgaatgtgcccatcattgcgctgagccagctgtcccgtgcggtggaaaagcagggcaacaactcctcccaccgcccccagctgtccgacctgcgtgattccggttccatcgagcaggacgccgactgcgtgctgttcctctaccgtgattcttattacgccagccagaacccggacggtgccgaggtggacgccgacacggccgagtgcatcgtggccaaaaaccgccacggtgagaccagtaccgtgccgctgggctgggatggtgcccacacccgctttatggatgtggacttcaaacgctga

SEQ ID NO: 13 - DNA, 777 bp, Ruminococcus bicirculans
atgaagaatatgataaaaatatttgaaaatgacgaattcggaaaagtgagaacagtcattaaggacggcgaaccgtggcttgtaggaaaagatgttgcggaaattttagggtattccaacacaagggacgctctttcacgtcatgtggataccgaggataaaaccaccgtcgtgatttccgacagtggttcaaattacaagagcaagaccactattatcaatgaaagcggcttttacagcttagttctctcaagcaaaatgccgagagccaaagagttcaggcgttgggtgaccgccgaagtcctccccaccatcagacgcaccggcggctacgtttccaacgaggatatgttcatcaaaaactatctcccctttctcgacgagccataccgtgacctgttccgacttcaaatgaccattatcaacaagctgaatgaacgtatccgccacgatcagccgctggtggagtttgcgaatcaggtgtcaaataccgataatcttatcgacatgaacgcaatggcaaagcttgcgagagcggaaaatatccccgtcggcagaaacaagctttacggctggctgaaaggaaaaggtgtgcttatggcaaacaatctgccgtatcaggcttttatcgaccgcggatatttttccgtaaaggagtcggtgtttgaaactgcgactatgacaaagacttatcagcagacgtttgttacgggcagggggcagcagttcgtcataaatttgctgaagaaatattatgggaaggaggttttgcaataa

SEQ ID NO: 14 - DNA, 858 bp, Faecalibacterium prausnitzii
atctccaaactggaaaaaacgctgcgggcacggttcccgaaaacgcagcagggcgaactgctggccggggcggtgctggccttctgcctgccggtgggcacctttctgctcacaagcgccgtgtgccttctggcggcaaaaatcagcccctggctcggccttgccgtgcagatgttctggtgcgggcaggcgctggcggcaaagggacttgtgcaggagagccggaacgtttacaacaagctggtaaagcccgacctgcccgccgcccgcaaggccgtgagccgcatcgtggggcgggacaccgagaacctgaccgccgagggcgtgaccaaggctgccgtggagactgtggccgagaatgccagcgacggcgtgattgcgccgctgctgtacatgctgctgggcggcgcgccgctggcgctgacctacaaggccgtcaacaccatggacagcatggtgggctacaaaaacgagacctatctctacttcggccgggcggcggcaaagctggacgatatggcaaactacattcccagccgccttgccgccctgctgtgggcggcggctgctgccctgaccggcaacgatgccaaaggcgcgtggcgcatctggcggcgggaccggcgcaatcacgccagccccaacagcgcccagaccgaaagcgcctgcgccggtgcgctgggcgtgcagctggccgggccggcctactactttggcgaatactacccgaaacccaccatcggcgatgccctgcgccccattgagccgcaggacatcctgcgggccgaccgcatgatgtacgccgccagcattctggcgctggtgctcgggcttgtgatacgggggttcgttgtatga

SEQ ID NO: 15 - DNA, 945 bp, Faecalibacterium prausnitzii
atgaacagagaaacggtgaacatggtgcgcagtccgatttctgtggaggggaacatccggcttgttccgtattatccggcctacgatacagcacttgcgtggtatcaggatgcacagctctgcaaacaggtagataacagggacttcgtttatgatttgccgctgctgaagcggatgtatcattatctggacacacacggggaactgttttatattgagtatcggggtgtgctttgtggtgacgtcagcctgcggacgaccggcgagctggccatcgtcatctgcaaggagtaccagaataaacacatcgggcggaaggtcatcgaaaaaatgctggagctggctcgggaaaggggcttggcggagtgcttcgcgcacatctattctttcaatacccagtcgcagaaaatgtttgaatccattggctttgtcccacaggacgaagaacgctatatctacaaattgcaaaaaggagaaccgactatgacaaaactgactctggaagaaaagcaggagctcatccggatggcccttgcggccagggagagggcttacgtgccttacagcgactttatggtgggcgctgccctgcgcgccgaggatggccgtgtctttaccggctgccatgtggagaatgccgcctttacccccaccagctgcgccgagcgcaccgcgctgttcaaagccgtgagcgagggcgtgaccaaatttacggacatcgccgtggtaggctcccgccggggcgagatcaatcagcagatcacctcgccctgcggcgtctgccgtcaggcactgtttgagtttggcggcccggagctgaacgtcatcatggccaaaacgccggatgatttcatggagcgcagcatggatgagctgctgccctttggcttcggtccctccaatgtggcgggcaacaaggccgtggaagaggaagaaaaaggctga

SEQ ID NO: 16 - DNA, 1206 bp, Unknown
atgaggttattttttgatatggtatgtaacggcagggcattgcaaaatgtacaaatgtataaattgaatatggttttagatgtacacccctatgctattacagcaccgtcaaaaactggtggccgttggcagacatatgtaaaggaaggtgataagcgtaagattataagggcttcttcaaaggaaaaactaatggacaaattatatactgcctattttgttcaaaatggtgtttctggtatgaccatggacaagctttttctcgaatggttagcttataaggaatgtatcacaaatagtatgaatacgattcgcagacatgaacaacactggaaaaagtattttcaggatatttccccaaataaggtatcttcctatgatcgtctggaattgcagaaagaatgtaatcagttaataaaagttaataacctttcttccaaagaatggcagaatgtaaaaacaattcttttaggtatgtttgactatgcctttgaaaaaggatatattaatacaaaccccatgcccagtattaaaatcactgttaaattccgtcaggtcaataaaaagagtggtaggactgaaacatatcagacagacgaatacaaagcacttatgcaatatctagatgcagaatatacagctacagaagaccttgctttattggctgttaaatttgatttttttattggatgccgtgttgctgagttggtagctctcaagtggtgtgatgttgaaaatctacggcatttacatatttgtagggaagaggttaaagagtctgtccgtgttggtgatacctggaaagatgtttataccgtttcagagcatactaagacatatacagaccggtctataaatttagttcctaatgcgattgctattttaaatcatatccgtcttaaaatggcttataatgtatctgacgatgattatatctttacccggaacggttcccggatcacttcacgccagattaattatattcttgaaaaagcatgtacaaaactgggaattatgattaagaggtcgcataaggtaagaaaaacggttgcaagtcgtctcaatgtcggtgaggttccgttagattctattcgtgagctgttaggtcatgcaaatttaagcactacactaagttatatttataatccgttatcggaaaaagaaacctataacctgatgtccagagccttggggaaagttcaatag

SEQ ID NO: 17 - DNA, 336 bp, Unknown
atggcgattgatactgaattagcaaaaagattacgttcatatcgtaattttaaacatttaacacaaaaagatgttgctgcgcatttaaatgttcctcattctgcaatttccgatatagaaaatggtaaaagagacattactgttagcgagttaaaagtgttttcaaatttatatggtagaagtgtagaagaaattatgagcgggaaaaaatatgactattataatattgccaatatcgctcgtttacttactgaacttcctgatgatgatttaaaagaaatcatgtttattattgaatataaaagaaaaagaaatgaagaacgtcatttgaaataa

SEQ ID NO: 18 - DNA, 816 bp, Treponema sp.
atggccaaaacacctatcgtagataaggggtgcttcatatcgaatgatgttaaaaggtcaatagttttaaacctatgtgagactaagtcaatggatctaattgcaagagaacactgtgtatctcctagtagtgttgccagaatacttcgtttaactgaagataggagaagaaaaaattatcttcctaggattctatcaatagacgaattcaagtcagtaaatacagttgatgcgtctatgagtgtaaatttaactgatttagaaggcggtcatatttttgatatcctggtggataggaggcaaagatacctctttgagtactttaattcctatcccttgaaggtcagaaaaagggtagaatatgtgactacagacatgtataagccatatattgatcttgccaagaaggtctttccaaatgccaatattgtggtagataaattccatatagtacagctcttgacaagagagctaaacaagttaaggataaatgagatgaagaagcttaataccaggtctagagagtataaaatactgaagagatactggaaaataccccttaggaagaagagagacttaaacagtatatatttttacaagaataggcactttaaaaatatgaccagttcaattgatatattagactatatgttaaaggaatttcccaacttaaaagaggcctatgatttttatcaaaacttcctattaagtatatctaataatgatgtcgctatgcttgaagacattctaaatactaggactgatgaaattcccatgtgttttaggaagagtataaaaagccttaaaaagcttaga

SEQ ID NO: 19 - DNA, 432 bp, Unknown
tatttttacaagaataggcactttaaaaatatgaccagttcagttgatatattagattatatgttaaaagaatttcccaacttaaaagatgcctatgatttttatcaaaacttcctattaagtatatctaataatgatgtggctatgcttgaagatattctaaatactaggactgataaaataccaatgtgttttaggaagagtataaaaagccttaaaaagtttagaaagtatgtggtaaattcactgaaatatgactatacgaatgccatggtggagggtaaaaacaacaagataaaggtaattaaaagagtatcctacggatataggagttttaggaattttaaggcaaggataatgctaatggaaaggtataaaatacaaaagggcaacatccatagttatcagtttgctatggatgctgccgcataa

SEQ ID NO: 20 - DNA, 873 bp, Unknown
atgaaacgtattttattaactggagcaagtggatttataggtaaaaacattaaagagacattaaacagtaaatatgacatatggagcccgtcaagccaggagctggatttaaaagataccgaatgcgttgaagcatatttgaagcagcattctttcgatgtaatattgcatgcagcaaattgtaatgatacaaggaattccatatcagcatacgatgtactcaatggaaatctcagaatgttttttaacctagagagatgttctcactattatggaaaaatgatttattttgggtctggggcagaatatgacagaagtaataacatccctaatatgtcagaggactattttgataccagtgttccgaaagatgcttacggactttcaaaatatattatggcaaaagcctgtttaaatcagaagaacatttatgaattgtgtttatttggagtatacggaaaatatgaggaatgggagagaagatttatctctaatgcgatatgtcgtgcattaaagggtatggatattacgcttcataaaaatgtatactttgattatttgtgggtagatgacctcataaaaattatttcttttttcattgagaaagataacttgaggtacaagaggtacaatgtgtgtagaggcgagaaggttgatctatattcgctggcagtacaggtaaagaagactttggatagcgaatgttcaatattagttggtgagcctggatggaagagggagtatactgcggataacaatagaatgttgaacgaaatgaatggtttatcttttacaaaactggaagtgacgatagctgaattgtgtgaatattataaagagcatttatcagaaatagttactgaaaaattgtaa